European Patent Application EP 4 644 412 A1, published November 5, 2025. Title: Platform for recombinant proteins using elastin like/based polypeptide and it's expression in animal cells. Applicant: NexThera Co.,Ltd. The sequence listing filed with the application follows.

SEQUENCE LISTING (19 sequences)

SEQ ID NO: 1 - protein, 30 aa, synthetic construct
VPAXGVPAXGVPAXGVPAXGVPAXGVPAXG

SEQ ID NO: 2 - protein, 30 aa, synthetic construct
VPGXGVPGXGVPGXGVPGXGVPGXGVPGXG

SEQ ID NO: 3 - protein, 90 aa, synthetic construct
VPAGGVPAAGVPAGGVPAGGVPAIGVPAGGVPAGGVPAAGVPAGGVPAGGVPAIGVPAGGVPAGGVPAAGVPAGGVPAGGVPAIGVPAGG

SEQ ID NO: 4 - protein, 180 aa, synthetic construct
VPAGGVPAAGVPAGGVPAGGVPAIGVPAGGVPAGGVPAAGVPAGGVPAGGVPAIGVPAGGVPAGGVPAAGVPAGGVPAGGVPAIGVPAGGVPAGGVPAAGVPAGGVPAGGVPAIGVPAGGVPAGGVPAAGVPAGGVPAGGVPAIGVPAGGVPAGGVPAAGVPAGGVPAGGVPAIGVPAGG

SEQ ID NO: 5 - protein, 360 aa, synthetic construct
VPAGGVPAAGVPAGGVPAGGVPAIGVPAGGVPAGGVPAAGVPAGGVPAGGVPAIGVPAGGVPAGGVPAAGVPAGGVPAGGVPAIGVPAGGVPAGGVPAAGVPAGGVPAGGVPAIGVPAGGVPAGGVPAAGVPAGGVPAGGVPAIGVPAGGVPAGGVPAAGVPAGGVPAGGVPAIGVPAGGVPAGGVPAAGVPAGGVPAGGVPAIGVPAGGVPAGGVPAAGVPAGGVPAGGVPAIGVPAGGVPAGGVPAAGVPAGGVPAGGVPAIGVPAGGVPAGGVPAAGVPAGGVPAGGVPAIGVPAGGVPAGGVPAAGVPAGGVPAGGVPAIGVPAGGVPAGGVPAAGVPAGGVPAGGVPAIGVPAGG

SEQ ID NO: 6 - protein, 90 aa, synthetic construct
VPGGGVPGAGVPGGGVPGGGVPGIGVPGGGVPGGGVPGAGVPGGGVPGGGVPGIGVPGGGVPGGGVPGAGVPGGGVPGGGVPGIGVPGGG

SEQ ID NO: 7 - protein, 180 aa, synthetic construct
VPGGGVPGAGVPGGGVPGGGVPGIGVPGGGVPGGGVPGAGVPGGGVPGGGVPGIGVPGGGVPGGGVPGAGVPGGGVPGGGVPGIGVPGGGVPGGGVPGAGVPGGGVPGGGVPGIGVPGGGVPGGGVPGAGVPGGGVPGGGVPGIGVPGGGVPGGGVPGAGVPGGGVPGGGVPGIGVPGGG

SEQ ID NO: 8 - protein, 360 aa, synthetic construct
VPGGGVPGAGVPGGGVPGGGVPGIGVPGGGVPGGGVPGAGVPGGGVPGGGVPGIGVPGGGVPGGGVPGAGVPGGGVPGGGVPGIGVPGGGVPGGGVPGAGVPGGGVPGGGVPGIGVPGGGVPGGGVPGAGVPGGGVPGGGVPGIGVPGGGVPGGGVPGAGVPGGGVPGGGVPGIGVPGGGVPGGGVPGAGVPGGGVPGGGVPGIGVPGGGVPGGGVPGAGVPGGGVPGGGVPGIGVPGGGVPGGGVPGAGVPGGGVPGGGVPGIGVPGGGVPGGGVPGAGVPGGGVPGGGVPGIGVPGGGVPGGGVPGAGVPGGGVPGGGVPGIGVPGGGVPGGGVPGAGVPGGGVPGGGVPGIGVPGGG

SEQ ID NO: 9 - protein, 235 aa, synthetic construct
EPRGPTIKPSPPSKSPAPNLLGGSSVFIFPPKIKDVLMISLSPIVTCVVVDVSEDDPDVQISWFVNNVEVHTAQTQTHREDYNSTLRVVSALPIQHQDWMSGKEFKCKVNNKDLPAPIERTISKPKGSVRAPQVYVLPPPEEEMTKKQATLTCMVTDFMPEDIYVEWTNNGKTELNYKNTEPVLDSDGSYFMYSKLRVEKKNWVERNSYSCSVVHEGLHNHHTTKSFSRTPGKTS

SEQ ID NO: 10 - protein, 227 aa, synthetic construct
DKTHTSPPSPAPELLGGPSVFLFPPKPKDTLMISRTPEVTCVVVDVSHEDPEVKFNWYVDGVEVHNAKTKPREEQYNSTYRVVSVLTVLHQDWLNGKEYKCKVSNKALPAPIEKTISKAKGQPREPQVYTLPPSRDELTKNQVSLTCLVKGFYPSDIAVEWESNGQPENNYKTTPPVLDSDGSFFLYSKLTVDKSRWQQGNVFSCSVMHEALHNHYTQKSLSLSPGK

SEQ ID NO: 11 - protein, 227 aa, synthetic construct
DKTHTCPPCPAPELLGGPSVFLFPPKPKDTLMISRTPEVTCVVVDVSHEDPEVKFNWYVDGVEVHNAKTKPREEQYNSTYRVVSVLTVLHQDWLNGKEYKCKVSNKALPAPIEKTISKAKGQPREPQVYTLPPSRDELTKNQVSLTCLVKGFYPSDIAVEWESNGQPENNYKTTPPVLDSDGSFFLYSKLTVDKSRWQQGNVFSCSVMHEALHNHYTQKSLSLSPGK

SEQ ID NO: 12 - protein, 223 aa, synthetic construct
VESPPSPAPPVAGPSVFLFPPKPKDTLMISRTPEVTCVVVDVSHEDPEVQFNWYVDGMEVHNAKTKPREEQFNSTFRVVSVLTVVHQDWLNGKEYKCKVSNKGLPAPIEKTISKTKGQPREPQVYTLPPSREEMTKNQVSLTCLVKGFYPSDIAVEWESNGQPENNYKTTPPMLDSDGSFFLYSKLTVDKSRWQQGNVFSCSVMHEALHNHYTQKSLSLSPGK

SEQ ID NO: 13 - protein, 6 aa, synthetic construct
GNQWFI

SEQ ID NO: 14 - protein, 14 aa, synthetic construct
IEGPTLRQWLAARA

SEQ ID NO: 15 - protein, 166 aa, synthetic construct
MSYNLLGFLQRSSNFQCQKLLWQLNGRLEYCLKDRMNFDIPEEIKQLQQFQKEDAALTIYEMLQNIFAIFRQDSSSTGWNETIVENLLANVYHQINHLKTVLEEKLEKEDFTRGKLMSSLHLKRYYGRILHYLKAKEYSHCAWTIVRVEILRNFYFINRLTGYLRN

SEQ ID NO: 16 - protein, 482 aa, synthetic construct
IDETRAHLLLKEKMMRLGGRLVLNTKEELANERLMTLKIAEMKEAMRTLIFPPSMHFFQAKHLIERSQVFNILRMMPKGAALHLHDIGIVTMDWLVRNVTYRPHCHICFTPRGIMQFRFAHPTPRPSEKCSKWILLEDYRKRVQNVTEFDDSLLRNFTLVTQHPEVIYTNQNVVWSKFETIFFTISGLIHYAPVFRDYVFRSMQEFYEDNVLYMEIRARLLPVYELSGEHHDEEWSVKTYQEVAQKFVETHPEFIGIKIIYSDHRSKDVAVIAESIRMAMGLRIKFPTVVAGFDLVGHEDTGHSLHDYKEALMIPAKDGVKLPYFFHAGETDWQGTSIDRNILDALMLNTTRIGHGFALSKHPAVRTYSWKKDIPIEVCPISNQVLKLVSDLRNHPVATLMATGHPMVISSDDPAMFGAKGLSYDFYEVFMGIGGMKADLRTLKQLAMNSIKYSTLLESEKNTFMEIWKKRWDKFIADVATK

SEQ ID NO: 17 - protein, 245 aa, synthetic construct
DIQMTQSPATLSVTPGDSVSLSCRASQSISKNLHWYQQKSHESPRLLIKFASQSISGIPSRFSGSGSGTDFTLSINSVETEDFGMYFCQQSNNWPLTFGAGTKLELKSSGGGGSGGGGGGSSRSSLEVQLKQSGPGLVKPSQSLSLTCSVTGYSFTSYYYWNWIRQFPGNRLEWMGYISYDGTNYYNPSLKNRISITRDTSKNQFFLNLNSMTTEDTATYYCAREENWDWYFDVWGAGTTVTVSS

SEQ ID NO: 18 - protein, 241 aa, synthetic construct
EVQLVESGGGLVQPGGSLRLSCAASGFTFSDSWIHWVRQAPGKGLEWVAWISPYGGSTYYADSVKGRFTISADTSKNTAYLQMNSLRAEDTAVYYCARRHWPGGFDYWGQGTLVTVSSGVGGSGGGGSGGGGSDIQMTQSPSSLSASVGDRVTITCRASQDVSTAVAWYQQKPGKAPKLLIYSASFLYSGVPSRFSGSGSGTDFTLTISSLQPEDFATYYCQQYLYHPATFGQGTKVEIKR

SEQ ID NO: 19 - protein, 244 aa, synthetic construct
MQVQLKQSGPGLVQPSQSLSITCTVSGFSLTNYGVHWVRQSPGKGLEWLGVIWSGGNTDYNTPFTSRLSINKDNSKSQVFFKMNSLQSNDTAIYYCARALTYYDYEFAYWGQGTLVTVSAKLGGGGSGGGGSGGGGSDILLTQSPVILSVSPGERVSFSCRASQSIGTNIHWYQQRTNGSPRLLIKYASESISGIPSRFSGSGSGTDFTLSINSVESEDIADYYCQQNNNWPTTFGAGTKLELK